European Patent Specification EP 3 690 044 B1, published January 10, 2024. Title: CRISPR ENABLED MULTIPLEXED GENOME ENGINEERING. Applicant: The Regents of the University of Colorado, A Body Corporate. Application Not Yet Assigned. The sequence listing filed with the application follows.

SEQUENCE LISTING (33 sequences)

SEQ ID NO: 1 - DNA, 22 bp, artificial sequence
  synthetic polynucleotide
ccgtggatcctaggctggtctc

SEQ ID NO: 2 - DNA, 17 bp, artificial sequence
  synthetic polynucleotide
gcctggctaagtgaatt

SEQ ID NO: 3 - DNA, 17 bp, artificial sequence
  synthetic polynucleotide
agcaaaaacaggtatta

SEQ ID NO: 4 - DNA, 17 bp, artificial sequence
  synthetic polynucleotide
aaacaggtattaaagag

SEQ ID NO: 5 - DNA, 17 bp, artificial sequence
  synthetic polynucleotide
gcctggccgcgtgaatt

SEQ ID NO: 6 - DNA, 17 bp, artificial sequence
  synthetic polynucleotide
ccagtttcaaggctgta

SEQ ID NO: 7 - DNA, 17 bp, Artificial Sequence
  synthetic polynucleotide
ccagtttgtaggctgta

SEQ ID NO: 8 - DNA, 17 bp, artificial sequence
  synthetic polynucleotide
cttcaaacgtaccctgg

SEQ ID NO: 9 - DNA, 17 bp, artificial sequence
  synthetic polynucleotide
agccaaaaataggtatt

SEQ ID NO: 10 - DNA, 17 bp, artificial sequence
  synthetic polynucleotide
gcctggccgcgtgaatt

SEQ ID NO: 11 - DNA, 17 bp, artificial sequence
  synthetic polynucleotide
cttcaaaaggaccctgg

SEQ ID NO: 12 - DNA, 17 bp, artificial sequence
  synthetic polynucleotide
cttcaaaacaaccctgg

SEQ ID NO: 13 - DNA, 1052 bp, artificial sequence
  synthetic polynucleotide
  misc_feature (325)..(325): n is a, c, g, or t
  misc_feature (632)..(632): n is a, c, g, or t
  misc_feature (806)..(806): n is a, c, g, or t
  misc_feature (892)..(892): n is a, c, g, or t
  misc_feature (985)..(985): n is a, c, g, or t
cggaaccggtattgcagcagctttatcatctgccgctggacggcgcacaaatcgcgcttaacggtcaggaagaacctcgtgaatcgcatctccgcaacgccaatgacactccgccagcagaacgcggcgttggtatggtgtttcagtcttacgcgctctatccccacctgtcagtagcagaaaacatgtcatttggcctgaaactggcaagcacgcccggtagcagagcccgagtattacatcgaactggatttcaacagcggtaagatccttgagagttttcgccccgaagaacgttttccaatgatgagcacttttaaagttntgctatgtggcgcggacggtttgggcgaggatgttcgggactgagcgtatggaagagcacttgcgttttgccgcctgctactggcacaccttctgctggaacggggcggatatgtttttcagattgggttgcgagtggtgggcgacggttttatgattgcaggtccgctgggcggctggtgcattaagcacttcgaccgctgggtagacggtaagatcaaatgccgattgtcagttggagggagcaagggaaccagatcaaaccagagcacttcaaaaactgggttgaatgggcgaaagccaatcanctcggtctggatccaaccatgcgtatcgtgccaagtgcgtcccagacaacaagtatatgaattatcggaggttgtcgatcaactcgatatacccgtactttgttatggtttacgtaccgattttcgaggtgaattatttattggcagcccccgttgtggtgtccttctgatgancccattacaggcacgcttgagccaggacctggcgcgcgagcaaattcgccaggcgcaggatggtcacttaccgacttgcaacttancccgctgttcccgaggacgttaacgcgctggtcgatgagtacaaaagctgctacaccatgacgccttgcataggagccacgaaccgccatacnagacattttgaggcatttcagtcagttgctcaatgtacctatacccagaccgttcagctggatatta

SEQ ID NO: 14 - DNA, 59 bp, artificial sequence
  synthetic polynucleotide
tttataaatagatggccaatacctccagtcctatggagttggaatgttaatgacccggg

SEQ ID NO: 15 - DNA, 59 bp, artificial sequence
  synthetic polynucleotide
tttataaatagatggccaatacctcaagggctttggagttggaatgttaatgacccggg

SEQ ID NO: 16 - DNA, 59 bp, artificial sequence
  synthetic polynucleotide
tttataaatagatggccaatacctcaaggcctatggagttggaatgttaatgacccggg

SEQ ID NO: 17 - DNA, 59 bp, artificial sequence
  synthetic polynucleotide
aaatatttatgtaccggttatggagttccggatacctcaaccttacaattactgggccc

SEQ ID NO: 18 - DNA, 76 bp, artificial sequence
  synthetic polynucleotide
cactcacaccatttaaacgcctggccgcgtgaatttgattggtgaacacaccgactacaacgacggtttcgttctg

SEQ ID NO: 19 - DNA, 76 bp, artificial sequence
  synthetic polynucleotide
cagaacgaaaccgtcgttgtagtcggtgtgttcaccaatcaaattcacgcggccaggcgtttaaatggtgtgagtg

SEQ ID NO: 20 - DNA, 24 bp, artificial sequence
  synthetic polynucleotide
cacaccatttaaacgcctggccgc

SEQ ID NO: 21 - DNA, 24 bp, artificial sequence
  synthetic polynucleotide
cacaccatttaagcgcctggccgc

SEQ ID NO: 22 - DNA, 24 bp, artificial sequence
  synthetic polynucleotide
cacaccattcaggcgcctggccgc

SEQ ID NO: 23 - DNA, 45 bp, artificial sequence
  synthetic polynucleotide
ggaaccgtattgcagcagctttatcatctgccgctggacggcgca

SEQ ID NO: 24 - protein, 15 aa, artificial sequence
  synthetic polypeptide
GTVLQQLYHLPLDGA

SEQ ID NO: 25 - DNA, 45 bp, artificial sequence
  synthetic polynucleotide
ggaacggtattgcagcagctttaacatctgccgctggacggcgca

SEQ ID NO: 26 - protein, 7 aa, artificial sequence
  synthetic polypeptide
GTVLQQL

SEQ ID NO: 27 - protein, 7 aa, artificial sequence
  synthetic polypeptide
HLPLDGA

SEQ ID NO: 28 - DNA, 200 bp, artificial sequence
  synthetic polynucleotide
ttcggatcgcaggctgcaccgggttaagttcttccgcttcactggaagtcgcggtcggaacggtattgcagcagctttaacatctgccgctggacggcgcacaaatcgcgcttaacgggatcttgacagctagctcagtcctaggtataatactagtatgataaagctgctgcaatagttttagagctagaaatagcaag

SEQ ID NO: 29 - DNA, 31 bp, artificial sequence
  synthetic polynucleotide
ccagaaatcatccttagcgaaagctaaggat

SEQ ID NO: 30 - DNA, 36 bp, artificial sequence
  synthetic polynucleotide
gttttagagctagaaatagcaagttaaaataaggct

SEQ ID NO: 31 - DNA, 60 bp, artificial sequence
  synthetic polynucleotide
atcacgaggcagaatttcagataaaaaaaatccttagctttcgctaaggatgatttctgg

SEQ ID NO: 32 - DNA, 60 bp, artificial sequence
  synthetic polynucleotide
actttttcaagttgataacggactagccttattttaacttgctatttctagctctaaaac

SEQ ID NO: 33 - DNA, 200 bp, artificial sequence
  synthetic polynucleotide
cttgctatttctagctctaaaactattgcagcagctttatcatactagtattatacctaggactgagctagctgtcaagatcccgttaagcgcgatttgtgcgccgtccagcggcagatgttaaagctgctgcaataccgttccgaccgcgacttccagtgaagcggaagaacttaacccggtgcagcctgcgatccgaa